European Patent Application EP 4 450 625 A1, published October 23, 2024. Title: Antisense oligonucleotide targeting ANT1 mRNA or pre-mRNA. Applicant: NIPPON SHINYAKU CO., LTD. Application JP. The sequence listing filed with the application follows.

SEQUENCE LISTING (473 sequences)

SEQ ID NO: 1 - DNA, 20 bp, synthetic construct
  misc_feature 1..20: note = Synthetic
  source 1..20: mol_type = other DNA
tcctcccacttggcgtccag

SEQ ID NO: 2 - DNA, 20 bp, synthetic construct
  misc_feature 1..20: note = Synthetic
  source 1..20: mol_type = other DNA
agaagcagagcgggaggccc

SEQ ID NO: 3 - DNA, 20 bp, synthetic construct
  misc_feature 1..20: note = Synthetic
  source 1..20: mol_type = other DNA
ttccccacagctgtggtctg

SEQ ID NO: 4 - DNA, 20 bp, synthetic construct
  misc_feature 1..20: note = Synthetic
  source 1..20: mol_type = other DNA
gtggaggcttcctctactcg

SEQ ID NO: 5 - DNA, 20 bp, synthetic construct
  misc_feature 1..20: note = Synthetic
  source 1..20: mol_type = other DNA
aggaggaaagagtggaggtg

SEQ ID NO: 6 - DNA, 20 bp, synthetic construct
  misc_feature 1..20: note = Synthetic
  source 1..20: mol_type = other DNA
ggtgctgtctggcggttgag

SEQ ID NO: 7 - DNA, 20 bp, synthetic construct
  misc_feature 1..20: note = Synthetic
  source 1..20: mol_type = other DNA
ttcaaagctagcctctggct

SEQ ID NO: 8 - DNA, 20 bp, synthetic construct
  misc_feature 1..20: note = Synthetic
  source 1..20: mol_type = other DNA
ttagggccccccactgatga

SEQ ID NO: 9 - DNA, 20 bp, synthetic construct
  misc_feature 1..20: note = Synthetic
  source 1..20: mol_type = other DNA
ggcaggttcggtgtcacatg

SEQ ID NO: 10 - DNA, 20 bp, synthetic construct
  misc_feature 1..20: note = Synthetic
  source 1..20: mol_type = other DNA
agaggctgatgcattgttga

SEQ ID NO: 11 - DNA, 20 bp, synthetic construct
  misc_feature 1..20: note = Synthetic
  source 1..20: mol_type = other DNA
tggttgggcccccaggccag

SEQ ID NO: 12 - DNA, 20 bp, synthetic construct
  misc_feature 1..20: note = Synthetic
  source 1..20: mol_type = other DNA
gcagatgaccaggtagtggt

SEQ ID NO: 13 - DNA, 20 bp, synthetic construct
  misc_feature 1..20: note = Synthetic
  source 1..20: mol_type = other DNA
ggagagggcagatgaccagg

SEQ ID NO: 14 - DNA, 20 bp, synthetic construct
  misc_feature 1..20: note = Synthetic
  source 1..20: mol_type = other DNA
ggtgaaggagccagagttgg

SEQ ID NO: 15 - DNA, 20 bp, synthetic construct
  misc_feature 1..20: note = Synthetic
  source 1..20: mol_type = other DNA
gagacagagaggcttgttgg

SEQ ID NO: 16 - DNA, 20 bp, synthetic construct
  misc_feature 1..20: note = Synthetic
  source 1..20: mol_type = other DNA
attggagacagagaggcttg

SEQ ID NO: 17 - DNA, 20 bp, synthetic construct
  misc_feature 1..20: note = Synthetic
  source 1..20: mol_type = other DNA
ctgattggagacagagaggc

SEQ ID NO: 18 - DNA, 20 bp, synthetic construct
  misc_feature 1..20: note = Synthetic
  source 1..20: mol_type = other DNA
ggctgattggagacagagag

SEQ ID NO: 19 - DNA, 20 bp, synthetic construct
  misc_feature 1..20: note = Synthetic
  source 1..20: mol_type = other DNA
agagaaggctgagtatactt

SEQ ID NO: 20 - DNA, 20 bp, synthetic construct
  misc_feature 1..20: note = Synthetic
  source 1..20: mol_type = other DNA
accctggctccacacagcct

SEQ ID NO: 21 - DNA, 20 bp, synthetic construct
  misc_feature 1..20: note = Synthetic
  source 1..20: mol_type = other DNA
gcattgctgttggctaagag

SEQ ID NO: 22 - DNA, 20 bp, synthetic construct
  misc_feature 1..20: note = Synthetic
  source 1..20: mol_type = other DNA
ctgttgctgttgctggtggt

SEQ ID NO: 23 - DNA, 20 bp, synthetic construct
  misc_feature 1..20: note = Synthetic
  source 1..20: mol_type = other DNA
ggcccagagtttccgtgatg

SEQ ID NO: 24 - DNA, 20 bp, synthetic construct
  misc_feature 1..20: note = Synthetic
  source 1..20: mol_type = other DNA
ggagctaccgccctccagtg

SEQ ID NO: 25 - DNA, 20 bp, synthetic construct
  misc_feature 1..20: note = Synthetic
  source 1..20: mol_type = other DNA
catggcgtaagggtgtgcgt

SEQ ID NO: 26 - DNA, 20 bp, synthetic construct
  misc_feature 1..20: note = Synthetic
  source 1..20: mol_type = other DNA
aggacacctggctgtgaggt

SEQ ID NO: 27 - DNA, 20 bp, synthetic construct
  misc_feature 1..20: note = Synthetic
  source 1..20: mol_type = other DNA
gcctgcttggctgtaggaca

SEQ ID NO: 28 - DNA, 20 bp, synthetic construct
  misc_feature 1..20: note = Synthetic
  source 1..20: mol_type = other DNA
gaagagactggagggccatt

SEQ ID NO: 29 - DNA, 20 bp, synthetic construct
  misc_feature 1..20: note = Synthetic
  source 1..20: mol_type = other DNA
ccacggtggcaatgaccgtg

SEQ ID NO: 30 - DNA, 20 bp, synthetic construct
  misc_feature 1..20: note = Synthetic
  source 1..20: mol_type = other DNA
gaggccgttttgtagcctgc

SEQ ID NO: 31 - DNA, 20 bp, synthetic construct
  misc_feature 1..20: note = Synthetic
  source 1..20: mol_type = other DNA
ggctctctttccgtacggtg

SEQ ID NO: 32 - DNA, 20 bp, synthetic construct
  misc_feature 1..20: note = Synthetic
  source 1..20: mol_type = other DNA
gcgacccgggtttgtatccg

SEQ ID NO: 33 - DNA, 20 bp, synthetic construct
  misc_feature 1..20: note = Synthetic
  source 1..20: mol_type = other DNA
cgaggttcctcgatagcccg

SEQ ID NO: 34 - DNA, 20 bp, synthetic construct
  misc_feature 1..20: note = Synthetic
  source 1..20: mol_type = other DNA
tcccacggtgggcgagcccg

SEQ ID NO: 35 - DNA, 20 bp, synthetic construct
  misc_feature 1..20: note = Synthetic
  source 1..20: mol_type = other DNA
ggtggtggcagcgatggcag

SEQ ID NO: 36 - DNA, 20 bp, synthetic construct
  misc_feature 1..20: note = Synthetic
  source 1..20: mol_type = other DNA
cagcttggagccctccagtg

SEQ ID NO: 37 - DNA, 20 bp, synthetic construct
  misc_feature 1..20: note = Synthetic
  source 1..20: mol_type = other DNA
ctgctcggcctcgcgccgca

SEQ ID NO: 38 - DNA, 20 bp, synthetic construct
  misc_feature 1..20: note = Synthetic
  source 1..20: mol_type = other DNA
tcttcgcgcgcgcgctgctc

SEQ ID NO: 39 - DNA, 20 bp, synthetic construct
  misc_feature 1..20: note = Synthetic
  source 1..20: mol_type = other DNA
tctttctcgcgttcccgctc

SEQ ID NO: 40 - DNA, 20 bp, synthetic construct
  misc_feature 1..20: note = Synthetic
  source 1..20: mol_type = other DNA
tcaagctcgcgctccttctc

SEQ ID NO: 41 - DNA, 20 bp, synthetic construct
  misc_feature 1..20: note = Synthetic
  source 1..20: mol_type = other DNA
acgctgcgttcaagctcgcg

SEQ ID NO: 42 - DNA, 20 bp, synthetic construct
  misc_feature 1..20: note = Synthetic
  source 1..20: mol_type = other DNA
gcattccaccggagcacggc

SEQ ID NO: 43 - DNA, 20 bp, synthetic construct
  misc_feature 1..20: note = Synthetic
  source 1..20: mol_type = other DNA
cgcactgcccggttcaaatg

SEQ ID NO: 44 - DNA, 20 bp, synthetic construct
  misc_feature 1..20: note = Synthetic
  source 1..20: mol_type = other DNA
gcttcccgttccctctcccg

SEQ ID NO: 45 - DNA, 20 bp, synthetic construct
  misc_feature 1..20: note = Synthetic
  source 1..20: mol_type = other DNA
cacggaggtctcgttcacgg

SEQ ID NO: 46 - DNA, 20 bp, synthetic construct
  misc_feature 1..20: note = Synthetic
  source 1..20: mol_type = other DNA
gaaagggatccaagcccggc

SEQ ID NO: 47 - DNA, 20 bp, synthetic construct
  misc_feature 1..20: note = Synthetic
  source 1..20: mol_type = other DNA
gccaggctgcagagccaggc

SEQ ID NO: 48 - DNA, 20 bp, synthetic construct
  misc_feature 1..20: note = Synthetic
  source 1..20: mol_type = other DNA
ctagacgttctcgctccagg

SEQ ID NO: 49 - DNA, 20 bp, synthetic construct
  misc_feature 1..20: note = Synthetic
  source 1..20: mol_type = other DNA
gctggcccagctgccagcgc

SEQ ID NO: 50 - DNA, 20 bp, synthetic construct
  misc_feature 1..20: note = Synthetic
  source 1..20: mol_type = other DNA
gtgcaggtgcgagtggatgt

SEQ ID NO: 51 - DNA, 20 bp, synthetic construct
  misc_feature 1..20: note = Synthetic
  source 1..20: mol_type = other DNA
agaacttcgttctcgtgcag

SEQ ID NO: 52 - DNA, 20 bp, synthetic construct
  misc_feature 1..20: note = Synthetic
  source 1..20: mol_type = other DNA
gaggccggcaggtcccggta

SEQ ID NO: 53 - DNA, 20 bp, synthetic construct
  misc_feature 1..20: note = Synthetic
  source 1..20: mol_type = other DNA
gcagaaagggaggccggcag

SEQ ID NO: 54 - DNA, 20 bp, synthetic construct
  misc_feature 1..20: note = Synthetic
  source 1..20: mol_type = other DNA
gtgcatggcctgcagctgat

SEQ ID NO: 55 - DNA, 20 bp, synthetic construct
  misc_feature 1..20: note = Synthetic
  source 1..20: mol_type = other DNA
catgcagccactgctgctgt

SEQ ID NO: 56 - DNA, 20 bp, synthetic construct
  misc_feature 1..20: note = Synthetic
  source 1..20: mol_type = other DNA
gcagcggcacactgtgcagc

SEQ ID NO: 57 - DNA, 20 bp, synthetic construct
  misc_feature 1..20: note = Synthetic
  source 1..20: mol_type = other DNA
ccctccctcccccactctct

SEQ ID NO: 58 - DNA, 20 bp, synthetic construct
  misc_feature 1..20: note = Synthetic
  source 1..20: mol_type = other DNA
gccacctccccacctctgca

SEQ ID NO: 59 - DNA, 20 bp, synthetic construct
  misc_feature 1..20: note = Synthetic
  source 1..20: mol_type = other DNA
gcaggggacagccttgaagt

SEQ ID NO: 60 - DNA, 20 bp, synthetic construct
  misc_feature 1..20: note = Synthetic
  source 1..20: mol_type = other DNA
ctcgggccttcttggctgtc

SEQ ID NO: 61 - DNA, 20 bp, synthetic construct
  misc_feature 1..20: note = Synthetic
  source 1..20: mol_type = other DNA
ctcactttcactctctgaga

SEQ ID NO: 62 - DNA, 20 bp, synthetic construct
  misc_feature 1..20: note = Synthetic
  source 1..20: mol_type = other DNA
ggtctcctcactttcactct

SEQ ID NO: 63 - DNA, 20 bp, synthetic construct
  misc_feature 1..20: note = Synthetic
  source 1..20: mol_type = other DNA
ggtcgctgctgccatcatca

SEQ ID NO: 64 - DNA, 20 bp, synthetic construct
  misc_feature 1..20: note = Synthetic
  source 1..20: mol_type = other DNA
tagggtcgctgctgccatca

SEQ ID NO: 65 - DNA, 20 bp, synthetic construct
  misc_feature 1..20: note = Synthetic
  source 1..20: mol_type = other DNA
gggacgtgcttcggttgtcc

SEQ ID NO: 66 - DNA, 20 bp, synthetic construct
  misc_feature 1..20: note = Synthetic
  source 1..20: mol_type = other DNA
ctgtcgaggggtgctgtctg

SEQ ID NO: 67 - DNA, 20 bp, synthetic construct
  misc_feature 1..20: note = Synthetic
  source 1..20: mol_type = other DNA
tggctgtcgaggggtgctgt

SEQ ID NO: 68 - DNA, 20 bp, synthetic construct
  misc_feature 1..20: note = Synthetic
  source 1..20: mol_type = other DNA
aagctagcctctggctgtcg

SEQ ID NO: 69 - DNA, 20 bp, synthetic construct
  misc_feature 1..20: note = Synthetic
  source 1..20: mol_type = other DNA
gttcaaagctagcctctggc

SEQ ID NO: 70 - DNA, 20 bp, synthetic construct
  misc_feature 1..20: note = Synthetic
  source 1..20: mol_type = other DNA
ggggttcaaagctagcctct

SEQ ID NO: 71 - DNA, 20 bp, synthetic construct
  misc_feature 1..20: note = Synthetic
  source 1..20: mol_type = other DNA
atatccagtgggtgtcacag

SEQ ID NO: 72 - DNA, 20 bp, synthetic construct
  misc_feature 1..20: note = Synthetic
  source 1..20: mol_type = other DNA
ggaggagcctggaacattcg

SEQ ID NO: 73 - DNA, 20 bp, synthetic construct
  misc_feature 1..20: note = Synthetic
  source 1..20: mol_type = other DNA
ggtctcagggcaggtggggg

SEQ ID NO: 74 - DNA, 20 bp, synthetic construct
  misc_feature 1..20: note = Synthetic
  source 1..20: mol_type = other DNA
aggggtctcagggcaggtgg

SEQ ID NO: 75 - DNA, 20 bp, synthetic construct
  misc_feature 1..20: note = Synthetic
  source 1..20: mol_type = other DNA
ttgaggggtctcagggcagg

SEQ ID NO: 76 - DNA, 20 bp, synthetic construct
  misc_feature 1..20: note = Synthetic
  source 1..20: mol_type = other DNA
gcattgttgaggggtctcag

SEQ ID NO: 77 - DNA, 20 bp, synthetic construct
  misc_feature 1..20: note = Synthetic
  source 1..20: mol_type = other DNA
atgcattgttgaggggtctc

SEQ ID NO: 78 - DNA, 20 bp, synthetic construct
  misc_feature 1..20: note = Synthetic
  source 1..20: mol_type = other DNA
gggagaggctgatgcattgt

SEQ ID NO: 79 - DNA, 20 bp, synthetic construct
  misc_feature 1..20: note = Synthetic
  source 1..20: mol_type = other DNA
caggccagggggagaggctg

SEQ ID NO: 80 - DNA, 20 bp, synthetic construct
  misc_feature 1..20: note = Synthetic
  source 1..20: mol_type = other DNA
ccccaggccagggggagagg

SEQ ID NO: 81 - DNA, 20 bp, synthetic construct
  misc_feature 1..20: note = Synthetic
  source 1..20: mol_type = other DNA
ggcccccaggccagggggag

SEQ ID NO: 82 - DNA, 20 bp, synthetic construct
  misc_feature 1..20: note = Synthetic
  source 1..20: mol_type = other DNA
ttgggcccccaggccagggg

SEQ ID NO: 83 - DNA, 20 bp, synthetic construct
  misc_feature 1..20: note = Synthetic
  source 1..20: mol_type = other DNA
tgaccaggtagtggttgggc

SEQ ID NO: 84 - DNA, 20 bp, synthetic construct
  misc_feature 1..20: note = Synthetic
  source 1..20: mol_type = other DNA
gagagggcagatgaccaggt

SEQ ID NO: 85 - DNA, 20 bp, synthetic construct
  misc_feature 1..20: note = Synthetic
  source 1..20: mol_type = other DNA
ggggagagggcagatgacca

SEQ ID NO: 86 - DNA, 20 bp, synthetic construct
  misc_feature 1..20: note = Synthetic
  source 1..20: mol_type = other DNA
ccatggcgtggggagagggc

SEQ ID NO: 87 - DNA, 20 bp, synthetic construct
  misc_feature 1..20: note = Synthetic
  source 1..20: mol_type = other DNA
gtcccatggcgtggggagag

SEQ ID NO: 88 - DNA, 20 bp, synthetic construct
  misc_feature 1..20: note = Synthetic
  source 1..20: mol_type = other DNA
ccctgtcccatggcgtgggg

SEQ ID NO: 89 - DNA, 20 bp, synthetic construct
  misc_feature 1..20: note = Synthetic
  source 1..20: mol_type = other DNA
ggcccttctctgggccagga

SEQ ID NO: 90 - DNA, 20 bp, synthetic construct
  misc_feature 1..20: note = Synthetic
  source 1..20: mol_type = other DNA
gaagaggaggctgctgcaga

SEQ ID NO: 91 - DNA, 20 bp, synthetic construct
  misc_feature 1..20: note = Synthetic
  source 1..20: mol_type = other DNA
tgggcaatgcctgggaagct

SEQ ID NO: 92 - DNA, 20 bp, synthetic construct
  misc_feature 1..20: note = Synthetic
  source 1..20: mol_type = other DNA
agtatacttggggggctgat

SEQ ID NO: 93 - DNA, 20 bp, synthetic construct
  misc_feature 1..20: note = Synthetic
  source 1..20: mol_type = other DNA
cagcctgggatgggagagaa

SEQ ID NO: 94 - DNA, 20 bp, synthetic construct
  misc_feature 1..20: note = Synthetic
  source 1..20: mol_type = other DNA
taagaggcggccatagggag

SEQ ID NO: 95 - DNA, 20 bp, synthetic construct
  misc_feature 1..20: note = Synthetic
  source 1..20: mol_type = other DNA
ctgttggctaagaggcggcc

SEQ ID NO: 96 - DNA, 20 bp, synthetic construct
  misc_feature 1..20: note = Synthetic
  source 1..20: mol_type = other DNA
ttgctgttggctaagaggcg

SEQ ID NO: 97 - DNA, 20 bp, synthetic construct
  misc_feature 1..20: note = Synthetic
  source 1..20: mol_type = other DNA
tgggcattgctgttggctaa

SEQ ID NO: 98 - DNA, 20 bp, synthetic construct
  misc_feature 1..20: note = Synthetic
  source 1..20: mol_type = other DNA
ggatgggcattgctgttggc

SEQ ID NO: 99 - DNA, 20 bp, synthetic construct
  misc_feature 1..20: note = Synthetic
  source 1..20: mol_type = other DNA
cctggatgggcattgctgtt

SEQ ID NO: 100 - DNA, 20 bp, synthetic construct
  misc_feature 1..20: note = Synthetic
  source 1..20: mol_type = other DNA
gggcctggatgggcattgct

SEQ ID NO: 101 - DNA, 20 bp, synthetic construct
  misc_feature 1..20: note = Synthetic
  source 1..20: mol_type = other DNA
aaggggcctggatgggcatt

SEQ ID NO: 102 - DNA, 20 bp, synthetic construct
  misc_feature 1..20: note = Synthetic
  source 1..20: mol_type = other DNA
gggaaggggcctggatgggc

SEQ ID NO: 103 - DNA, 20 bp, synthetic construct
  misc_feature 1..20: note = Synthetic
  source 1..20: mol_type = other DNA
gaaatgctccaggaggaggg

SEQ ID NO: 104 - DNA, 20 bp, synthetic construct
  misc_feature 1..20: note = Synthetic
  source 1..20: mol_type = other DNA
gcaggtgtgctggccctggt

SEQ ID NO: 105 - DNA, 20 bp, synthetic construct
  misc_feature 1..20: note = Synthetic
  source 1..20: mol_type = other DNA
ggcaggtgtgctggccctgg

SEQ ID NO: 106 - DNA, 20 bp, synthetic construct
  misc_feature 1..20: note = Synthetic
  source 1..20: mol_type = other DNA
gggggcaggtgtgctggccc

SEQ ID NO: 107 - DNA, 20 bp, synthetic construct
  misc_feature 1..20: note = Synthetic
  source 1..20: mol_type = other DNA
ggtgggggcaggtgtgctgg

SEQ ID NO: 108 - DNA, 20 bp, synthetic construct
  misc_feature 1..20: note = Synthetic
  source 1..20: mol_type = other DNA
tgaggtgggggcaggtgtgc

SEQ ID NO: 109 - DNA, 20 bp, synthetic construct
  misc_feature 1..20: note = Synthetic
  source 1..20: mol_type = other DNA
ctgtgaggtgggggcaggtg

SEQ ID NO: 110 - DNA, 20 bp, synthetic construct
  misc_feature 1..20: note = Synthetic
  source 1..20: mol_type = other DNA
tggctgtgaggtgggggcag

SEQ ID NO: 111 - DNA, 20 bp, synthetic construct
  misc_feature 1..20: note = Synthetic
  source 1..20: mol_type = other DNA
acctggctgtgaggtggggg

SEQ ID NO: 112 - DNA, 20 bp, synthetic construct
  misc_feature 1..20: note = Synthetic
  source 1..20: mol_type = other DNA
ttggctgtaggacacctggc

SEQ ID NO: 113 - DNA, 20 bp, synthetic construct
  misc_feature 1..20: note = Synthetic
  source 1..20: mol_type = other DNA
tgcttggctgtaggacacct

SEQ ID NO: 114 - DNA, 20 bp, synthetic construct
  misc_feature 1..20: note = Synthetic
  source 1..20: mol_type = other DNA
attggggcctgcttggctgt

SEQ ID NO: 115 - DNA, 20 bp, synthetic construct
  misc_feature 1..20: note = Synthetic
  source 1..20: mol_type = other DNA
ggcgccccttgagggccctg

SEQ ID NO: 116 - DNA, 20 bp, synthetic construct
  misc_feature 1..20: note = Synthetic
  source 1..20: mol_type = other DNA
tggcgaggaagccacggtgg

SEQ ID NO: 117 - DNA, 20 bp, synthetic construct
  misc_feature 1..20: note = Synthetic
  source 1..20: mol_type = other DNA
gctggcgaggaagccacggt

SEQ ID NO: 118 - DNA, 20 bp, synthetic construct
  misc_feature 1..20: note = Synthetic
  source 1..20: mol_type = other DNA
ggcccaggtggggaggccgt

SEQ ID NO: 119 - DNA, 20 bp, synthetic construct
  misc_feature 1..20: note = Synthetic
  source 1..20: mol_type = other DNA
gcccccggggacggggctct

SEQ ID NO: 120 - DNA, 20 bp, synthetic construct
  misc_feature 1..20: note = Synthetic
  source 1..20: mol_type = other DNA
agcccggtggggtccccgtt

SEQ ID NO: 121 - DNA, 20 bp, synthetic construct
  misc_feature 1..20: note = Synthetic
  source 1..20: mol_type = other DNA
agcccggcttgaaggtccct

SEQ ID NO: 122 - DNA, 20 bp, synthetic construct
  misc_feature 1..20: note = Synthetic
  source 1..20: mol_type = other DNA
gtggcaggggcccaggtccc

SEQ ID NO: 123 - DNA, 20 bp, synthetic construct
  misc_feature 1..20: note = Synthetic
  source 1..20: mol_type = other DNA
caggcctgagggccccgcag

SEQ ID NO: 124 - DNA, 20 bp, synthetic construct
  misc_feature 1..20: note = Synthetic
  source 1..20: mol_type = other DNA
ctcaggggcggccctgaggc

SEQ ID NO: 125 - DNA, 20 bp, synthetic construct
  misc_feature 1..20: note = Synthetic
  source 1..20: mol_type = other DNA
ggcccgcttcttggccagct

SEQ ID NO: 126 - DNA, 20 bp, synthetic construct
  misc_feature 1..20: note = Synthetic
  source 1..20: mol_type = other DNA
cgcaccttctccaccaggtc

SEQ ID NO: 127 - DNA, 20 bp, synthetic construct
  misc_feature 1..20: note = Synthetic
  source 1..20: mol_type = other DNA
cgctccttttcttcgcgcgc

SEQ ID NO: 128 - DNA, 20 bp, synthetic construct
  misc_feature 1..20: note = Synthetic
  source 1..20: mol_type = other DNA
cgctctttctcgcgttcccg

SEQ ID NO: 129 - DNA, 20 bp, synthetic construct
  misc_feature 1..20: note = Synthetic
  source 1..20: mol_type = other DNA
tcgcgctctttctcgcgttc

SEQ ID NO: 130 - DNA, 20 bp, synthetic construct
  misc_feature 1..20: note = Synthetic
  source 1..20: mol_type = other DNA
cgctcgcgctctttctcgcg

SEQ ID NO: 131 - DNA, 20 bp, synthetic construct
  misc_feature 1..20: note = Synthetic
  source 1..20: mol_type = other DNA
tcgcgctcgcgctctttctc

SEQ ID NO: 132 - DNA, 20 bp, synthetic construct
  misc_feature 1..20: note = Synthetic
  source 1..20: mol_type = other DNA
ttctcgcgctcgcgctcttt

SEQ ID NO: 133 - DNA, 20 bp, synthetic construct
  misc_feature 1..20: note = Synthetic
  source 1..20: mol_type = other DNA
tccttctcgcgctcgcgctc

SEQ ID NO: 134 - DNA, 20 bp, synthetic construct
  misc_feature 1..20: note = Synthetic
  source 1..20: mol_type = other DNA
cgctccttctcgcgctcgcg

SEQ ID NO: 135 - DNA, 20 bp, synthetic construct
  misc_feature 1..20: note = Synthetic
  source 1..20: mol_type = other DNA
tcgcgctccttctcgcgctc

SEQ ID NO: 136 - DNA, 20 bp, synthetic construct
  misc_feature 1..20: note = Synthetic
  source 1..20: mol_type = other DNA
agctcgcgctccttctcgcg

SEQ ID NO: 137 - DNA, 20 bp, synthetic construct
  misc_feature 1..20: note = Synthetic
  source 1..20: mol_type = other DNA
gagccaacttcacgctgcgt

SEQ ID NO: 138 - DNA, 20 bp, synthetic construct
  misc_feature 1..20: note = Synthetic
  source 1..20: mol_type = other DNA
tgggcccagagatgggcatt

SEQ ID NO: 139 - DNA, 20 bp, synthetic construct
  misc_feature 1..20: note = Synthetic
  source 1..20: mol_type = other DNA
caccgcactgcccggttcaa

SEQ ID NO: 140 - DNA, 20 bp, synthetic construct
  misc_feature 1..20: note = Synthetic
  source 1..20: mol_type = other DNA
agccaccgcactgcccggtt

SEQ ID NO: 141 - DNA, 20 bp, synthetic construct
  misc_feature 1..20: note = Synthetic
  source 1..20: mol_type = other DNA
tgtagccaccgcactgcccg

SEQ ID NO: 142 - DNA, 20 bp, synthetic construct
  misc_feature 1..20: note = Synthetic
  source 1..20: mol_type = other DNA
cactgtagccaccgcactgc

SEQ ID NO: 143 - DNA, 20 bp, synthetic construct
  misc_feature 1..20: note = Synthetic
  source 1..20: mol_type = other DNA
gggcactgtagccaccgcac

SEQ ID NO: 144 - DNA, 20 bp, synthetic construct
  misc_feature 1..20: note = Synthetic
  source 1..20: mol_type = other DNA
gtaggggggcactgtagcca

SEQ ID NO: 145 - DNA, 20 bp, synthetic construct
  misc_feature 1..20: note = Synthetic
  source 1..20: mol_type = other DNA
ggtccactgcccccaggggc

SEQ ID NO: 146 - DNA, 20 bp, synthetic construct
  misc_feature 1..20: note = Synthetic
  source 1..20: mol_type = other DNA
ggggttccagctcactaggc

SEQ ID NO: 147 - DNA, 20 bp, synthetic construct
  misc_feature 1..20: note = Synthetic
  source 1..20: mol_type = other DNA
aaagggtgcaggccaggtgg

SEQ ID NO: 148 - DNA, 20 bp, synthetic construct
  misc_feature 1..20: note = Synthetic
  source 1..20: mol_type = other DNA
gcctctcagctgccagccgc

SEQ ID NO: 149 - DNA, 20 bp, synthetic construct
  misc_feature 1..20: note = Synthetic
  source 1..20: mol_type = other DNA
ccagggccgccaccctttct

SEQ ID NO: 150 - DNA, 20 bp, synthetic construct
  misc_feature 1..20: note = Synthetic
  source 1..20: mol_type = other DNA
taaggggcagcaaagagctg

SEQ ID NO: 151 - DNA, 20 bp, synthetic construct
  misc_feature 1..20: note = Synthetic
  source 1..20: mol_type = other DNA
tgagctgctgacatcggggc

SEQ ID NO: 152 - DNA, 20 bp, synthetic construct
  misc_feature 1..20: note = Synthetic
  source 1..20: mol_type = other DNA
agctcagctgactgtgcgtg

SEQ ID NO: 153 - DNA, 20 bp, synthetic construct
  misc_feature 1..20: note = Synthetic
  source 1..20: mol_type = other DNA
gttccagcgccaagcgctgc

SEQ ID NO: 154 - DNA, 20 bp, synthetic construct
  misc_feature 1..20: note = Synthetic
  source 1..20: mol_type = other DNA
ctcctgggcaggcagcggca

SEQ ID NO: 155 - DNA, 20 bp, synthetic construct
  misc_feature 1..20: note = Synthetic
  source 1..20: mol_type = other DNA
caggccaagggcacggtggg

SEQ ID NO: 156 - DNA, 20 bp, synthetic construct
  misc_feature 1..20: note = Synthetic
  source 1..20: mol_type = other DNA
tggccttctgtctgtccctc

SEQ ID NO: 157 - DNA, 20 bp, synthetic construct
  misc_feature 1..20: note = Synthetic
  source 1..20: mol_type = other DNA
ctgcacaccacatcgggcct

SEQ ID NO: 158 - DNA, 20 bp, synthetic construct
  misc_feature 1..20: note = Synthetic
  source 1..20: mol_type = other DNA
gtccccatcctcgccacctc

SEQ ID NO: 159 - DNA, 20 bp, synthetic construct
  misc_feature 1..20: note = Synthetic
  source 1..20: mol_type = other DNA
aatcacaccaacggggcagg

SEQ ID NO: 160 - DNA, 20 bp, synthetic construct
  misc_feature 1..20: note = Synthetic
  source 1..20: mol_type = other DNA
tggcacacgatgctacgcaa

SEQ ID NO: 161 - DNA, 20 bp, synthetic construct
  misc_feature 1..20: note = Synthetic
  source 1..20: mol_type = other DNA
gggtggcacacgatgctacg

SEQ ID NO: 162 - DNA, 20 bp, synthetic construct
  misc_feature 1..20: note = Synthetic
  source 1..20: mol_type = other DNA
caggggtggcacacgatgct

SEQ ID NO: 163 - DNA, 20 bp, synthetic construct
  misc_feature 1..20: note = Synthetic
  source 1..20: mol_type = other DNA
gggcaggggtggcacacgat

SEQ ID NO: 164 - DNA, 20 bp, synthetic construct
  misc_feature 1..20: note = Synthetic
  source 1..20: mol_type = other DNA
ctactcgggccttcttggct

SEQ ID NO: 165 - DNA, 20 bp, synthetic construct
  misc_feature 1..20: note = Synthetic
  source 1..20: mol_type = other DNA
cctctactcgggccttcttg

SEQ ID NO: 166 - DNA, 20 bp, synthetic construct
  misc_feature 1..20: note = Synthetic
  source 1..20: mol_type = other DNA
cttcctctactcgggccttc

SEQ ID NO: 167 - DNA, 20 bp, synthetic construct
  misc_feature 1..20: note = Synthetic
  source 1..20: mol_type = other DNA
ggctaagaggcggccatagg

SEQ ID NO: 168 - DNA, 20 bp, synthetic construct
  misc_feature 1..20: note = Synthetic
  source 1..20: mol_type = other DNA
gttggctaagaggcggccat

SEQ ID NO: 169 - DNA, 20 bp, synthetic construct
  misc_feature 1..20: note = Synthetic
  source 1..20: mol_type = other DNA
tgttggctaagaggcggcca

SEQ ID NO: 170 - DNA, 20 bp, synthetic construct
  misc_feature 1..20: note = Synthetic
  source 1..20: mol_type = other DNA
gctgttggctaagaggcggc

SEQ ID NO: 171 - DNA, 20 bp, synthetic construct
  misc_feature 1..20: note = Synthetic
  source 1..20: mol_type = other DNA
tgctgttggctaagaggcgg

SEQ ID NO: 172 - DNA, 20 bp, synthetic construct
  misc_feature 1..20: note = Synthetic
  source 1..20: mol_type = other DNA
attgctgttggctaagaggc

SEQ ID NO: 173 - DNA, 20 bp, synthetic construct
  misc_feature 1..20: note = Synthetic
  source 1..20: mol_type = other DNA
cattgctgttggctaagagg

SEQ ID NO: 174 - DNA, 20 bp, synthetic construct
  misc_feature 1..20: note = Synthetic
  source 1..20: mol_type = other DNA
ggcattgctgttggctaaga

SEQ ID NO: 175 - DNA, 20 bp, synthetic construct
  misc_feature 1..20: note = Synthetic
  source 1..20: mol_type = other DNA
gggcattgctgttggctaag

SEQ ID NO: 176 - DNA, 20 bp, synthetic construct
  misc_feature 1..20: note = Synthetic
  source 1..20: mol_type = other DNA
atgggcattgctgttggcta

SEQ ID NO: 177 - DNA, 20 bp, synthetic construct
  misc_feature 1..20: note = Synthetic
  source 1..20: mol_type = other DNA
gatgggcattgctgttggct

SEQ ID NO: 178 - DNA, 20 bp, synthetic construct
  misc_feature 1..20: note = Synthetic
  source 1..20: mol_type = other DNA
tggatgggcattgctgttgg

SEQ ID NO: 179 - DNA, 20 bp, synthetic construct
  misc_feature 1..20: note = Synthetic
  source 1..20: mol_type = other DNA
ctggatgggcattgctgttg

SEQ ID NO: 180 - DNA, 20 bp, synthetic construct
  misc_feature 1..20: note = Synthetic
  source 1..20: mol_type = other DNA
gcctggatgggcattgctgt

SEQ ID NO: 181 - DNA, 20 bp, synthetic construct
  misc_feature 1..20: note = Synthetic
  source 1..20: mol_type = other DNA
ggcctggatgggcattgctg

SEQ ID NO: 182 - DNA, 20 bp, synthetic construct
  misc_feature 1..20: note = Synthetic
  source 1..20: mol_type = other DNA
ggggcctggatgggcattgc

SEQ ID NO: 183 - DNA, 20 bp, synthetic construct
  misc_feature 1..20: note = Synthetic
  source 1..20: mol_type = other DNA
aggtgggggcaggtgtgctg

SEQ ID NO: 184 - DNA, 20 bp, synthetic construct
  misc_feature 1..20: note = Synthetic
  source 1..20: mol_type = other DNA
gaggtgggggcaggtgtgct

SEQ ID NO: 185 - DNA, 20 bp, synthetic construct
  misc_feature 1..20: note = Synthetic
  source 1..20: mol_type = other DNA
cgaggaagccacggtggcaa

SEQ ID NO: 186 - DNA, 20 bp, synthetic construct
  misc_feature 1..20: note = Synthetic
  source 1..20: mol_type = other DNA
ccttctccaccaggtcggcc

SEQ ID NO: 187 - DNA, 20 bp, synthetic construct
  misc_feature 1..20: note = Synthetic
  source 1..20: mol_type = other DNA
gcgccgcaccttctccacca

SEQ ID NO: 188 - DNA, 20 bp, synthetic construct
  misc_feature 1..20: note = Synthetic
  source 1..20: mol_type = other DNA
ctctttctcgcgttcccgct

SEQ ID NO: 189 - DNA, 20 bp, synthetic construct
  misc_feature 1..20: note = Synthetic
  source 1..20: mol_type = other DNA
gctctttctcgcgttcccgc

SEQ ID NO: 190 - DNA, 20 bp, synthetic construct
  misc_feature 1..20: note = Synthetic
  source 1..20: mol_type = other DNA
gcgctctttctcgcgttccc

SEQ ID NO: 191 - DNA, 20 bp, synthetic construct
  misc_feature 1..20: note = Synthetic
  source 1..20: mol_type = other DNA
cgcgctctttctcgcgttcc

SEQ ID NO: 192 - DNA, 20 bp, synthetic construct
  misc_feature 1..20: note = Synthetic
  source 1..20: mol_type = other DNA
ctcgcgctctttctcgcgtt

SEQ ID NO: 193 - DNA, 20 bp, synthetic construct
  misc_feature 1..20: note = Synthetic
  source 1..20: mol_type = other DNA
gctcgcgctctttctcgcgt

SEQ ID NO: 194 - DNA, 20 bp, synthetic construct
  misc_feature 1..20: note = Synthetic
  source 1..20: mol_type = other DNA
gcgctcgcgctctttctcgc

SEQ ID NO: 195 - DNA, 20 bp, synthetic construct
  misc_feature 1..20: note = Synthetic
  source 1..20: mol_type = other DNA
cgcgctcgcgctctttctcg

SEQ ID NO: 196 - DNA, 20 bp, synthetic construct
  misc_feature 1..20: note = Synthetic
  source 1..20: mol_type = other DNA
ctcgcgctcgcgctctttct

SEQ ID NO: 197 - DNA, 20 bp, synthetic construct
  misc_feature 1..20: note = Synthetic
  source 1..20: mol_type = other DNA
tctcgcgctcgcgctctttc

SEQ ID NO: 198 - DNA, 20 bp, synthetic construct
  misc_feature 1..20: note = Synthetic
  source 1..20: mol_type = other DNA
cttctcgcgctcgcgctctt

SEQ ID NO: 199 - DNA, 20 bp, synthetic construct
  misc_feature 1..20: note = Synthetic
  source 1..20: mol_type = other DNA
ccttctcgcgctcgcgctct

SEQ ID NO: 200 - DNA, 20 bp, synthetic construct
  misc_feature 1..20: note = Synthetic
  source 1..20: mol_type = other DNA
ctccttctcgcgctcgcgct

SEQ ID NO: 201 - DNA, 20 bp, synthetic construct
  misc_feature 1..20: note = Synthetic
  source 1..20: mol_type = other DNA
gctccttctcgcgctcgcgc

SEQ ID NO: 202 - DNA, 20 bp, synthetic construct
  misc_feature 1..20: note = Synthetic
  source 1..20: mol_type = other DNA
gcgctccttctcgcgctcgc

SEQ ID NO: 203 - DNA, 20 bp, synthetic construct
  misc_feature 1..20: note = Synthetic
  source 1..20: mol_type = other DNA
cgcgctccttctcgcgctcg

SEQ ID NO: 204 - DNA, 20 bp, synthetic construct
  misc_feature 1..20: note = Synthetic
  source 1..20: mol_type = other DNA
gcactgtagccaccgcactg

SEQ ID NO: 205 - DNA, 20 bp, synthetic construct
  misc_feature 1..20: note = Synthetic
  source 1..20: mol_type = other DNA
ggcactgtagccaccgcact

SEQ ID NO: 206 - DNA, 20 bp, synthetic construct
  misc_feature 1..20: note = Synthetic
  source 1..20: mol_type = other DNA
ggggcactgtagccaccgca

SEQ ID NO: 207 - DNA, 20 bp, synthetic construct
  misc_feature 1..20: note = Synthetic
  source 1..20: mol_type = other DNA
gggggcactgtagccaccgc

SEQ ID NO: 208 - DNA, 20 bp, synthetic construct
  misc_feature 1..20: note = Synthetic
  source 1..20: mol_type = other DNA
ggggggcactgtagccaccg

SEQ ID NO: 209 - DNA, 20 bp, synthetic construct
  misc_feature 1..20: note = Synthetic
  source 1..20: mol_type = other DNA
ccgggtccactgcccccagg

SEQ ID NO: 210 - DNA, 20 bp, synthetic construct
  misc_feature 1..20: note = Synthetic
  source 1..20: mol_type = other DNA
tgctgcctctcagctgccag

SEQ ID NO: 211 - DNA, 20 bp, synthetic construct
  misc_feature 1..20: note = Synthetic
  source 1..20: mol_type = other DNA
tgcgtgctgcctctcagctg

SEQ ID NO: 212 - DNA, 20 bp, synthetic construct
  misc_feature 1..20: note = Synthetic
  source 1..20: mol_type = other DNA
ctgctgacatcggggcagaa

SEQ ID NO: 213 - DNA, 20 bp, synthetic construct
  misc_feature 1..20: note = Synthetic
  source 1..20: mol_type = other DNA
ctgatgagctgctgacatcg

SEQ ID NO: 214 - DNA, 20 bp, synthetic construct
  misc_feature 1..20: note = Synthetic
  source 1..20: mol_type = other DNA
cagcgccaagcgctgcagct

SEQ ID NO: 215 - DNA, 20 bp, synthetic construct
  misc_feature 1..20: note = Synthetic
  source 1..20: mol_type = other DNA
tgctgttccagcgccaagcg

SEQ ID NO: 216 - DNA, 20 bp, synthetic construct
  misc_feature 1..20: note = Synthetic
  source 1..20: mol_type = other DNA
gggcaggcagcggcacactg

SEQ ID NO: 217 - DNA, 20 bp, synthetic construct
  misc_feature 1..20: note = Synthetic
  source 1..20: mol_type = other DNA
acaccacatcgggccttggc

SEQ ID NO: 218 - DNA, 20 bp, synthetic construct
  misc_feature 1..20: note = Synthetic
  source 1..20: mol_type = other DNA
acctctgcacaccacatcgg

SEQ ID NO: 219 - DNA, 20 bp, synthetic construct
  misc_feature 1..20: note = Synthetic
  source 1..20: mol_type = other DNA
gcaggggtggcacacgatgc

SEQ ID NO: 220 - DNA, 20 bp, synthetic construct
  misc_feature 1..20: note = Synthetic
  source 1..20: mol_type = other DNA
ggcaggggtggcacacgatg

SEQ ID NO: 221 - DNA, 20 bp, synthetic construct
  misc_feature 1..20: note = Synthetic
  source 1..20: mol_type = other DNA
ggggcaggggtggcacacga

SEQ ID NO: 222 - DNA, 20 bp, synthetic construct
  misc_feature 1..20: note = Synthetic
  source 1..20: mol_type = other DNA
gggcgcgcacacagggatcg

SEQ ID NO: 223 - DNA, 20 bp, synthetic construct
  misc_feature 1..20: note = Synthetic
  source 1..20: mol_type = other DNA
actcgggccttcttggctgt

SEQ ID NO: 224 - DNA, 20 bp, synthetic construct
  misc_feature 1..20: note = Synthetic
  source 1..20: mol_type = other DNA
tactcgggccttcttggctg

SEQ ID NO: 225 - DNA, 20 bp, synthetic construct
  misc_feature 1..20: note = Synthetic
  source 1..20: mol_type = other DNA
tctactcgggccttcttggc

SEQ ID NO: 226 - DNA, 20 bp, synthetic construct
  misc_feature 1..20: note = Synthetic
  source 1..20: mol_type = other DNA
ctctactcgggccttcttgg

SEQ ID NO: 227 - DNA, 20 bp, synthetic construct
  misc_feature 1..20: note = Synthetic
  source 1..20: mol_type = other DNA
tcctctactcgggccttctt

SEQ ID NO: 228 - DNA, 20 bp, synthetic construct
  misc_feature 1..20: note = Synthetic
  source 1..20: mol_type = other DNA
ttcctctactcgggccttct

SEQ ID NO: 229 - DNA, 20 bp, synthetic construct
  misc_feature 1..20: note = Synthetic
  source 1..20: mol_type = other DNA
gcttcctctactcgggcctt

SEQ ID NO: 230 - DNA, 20 bp, synthetic construct
  misc_feature 1..20: note = Synthetic
  source 1..20: mol_type = other DNA
ggcttcctctactcgggcct

SEQ ID NO: 231 - DNA, 20 bp, synthetic construct
  misc_feature 1..20: note = Synthetic
  source 1..20: mol_type = other DNA
ctaagaggcggccataggga

SEQ ID NO: 232 - DNA, 20 bp, synthetic construct
  misc_feature 1..20: note = Synthetic
  source 1..20: mol_type = other DNA
gctaagaggcggccataggg

SEQ ID NO: 233 - DNA, 20 bp, synthetic construct
  misc_feature 1..20: note = Synthetic
  source 1..20: mol_type = other DNA
tggctaagaggcggccatag

SEQ ID NO: 234 - DNA, 20 bp, synthetic construct
  misc_feature 1..20: note = Synthetic
  source 1..20: mol_type = other DNA
ttggctaagaggcggccata

SEQ ID NO: 235 - DNA, 20 bp, synthetic construct
  misc_feature 1..20: note = Synthetic
  source 1..20: mol_type = other DNA
gtgaggtgggggcaggtgtg

SEQ ID NO: 236 - DNA, 20 bp, synthetic construct
  misc_feature 1..20: note = Synthetic
  source 1..20: mol_type = other DNA
tgtgaggtgggggcaggtgt

SEQ ID NO: 237 - DNA, 20 bp, synthetic construct
  misc_feature 1..20: note = Synthetic
  source 1..20: mol_type = other DNA
gctgtgaggtgggggcaggt

SEQ ID NO: 238 - DNA, 20 bp, synthetic construct
  misc_feature 1..20: note = Synthetic
  source 1..20: mol_type = other DNA
ggctgtgaggtgggggcagg

SEQ ID NO: 239 - DNA, 20 bp, synthetic construct
  misc_feature 1..20: note = Synthetic
  source 1..20: mol_type = other DNA
ctggctgtgaggtgggggca

SEQ ID NO: 240 - DNA, 20 bp, synthetic construct
  misc_feature 1..20: note = Synthetic
  source 1..20: mol_type = other DNA
gaggaagccacggtggcaat

SEQ ID NO: 241 - DNA, 20 bp, synthetic construct
  misc_feature 1..20: note = Synthetic
  source 1..20: mol_type = other DNA
cggcccgcttcttggccagc

SEQ ID NO: 242 - DNA, 20 bp, synthetic construct
  misc_feature 1..20: note = Synthetic
  source 1..20: mol_type = other DNA
tcggcccgcttcttggccag

SEQ ID NO: 243 - DNA, 20 bp, synthetic construct
  misc_feature 1..20: note = Synthetic
  source 1..20: mol_type = other DNA
gtcggcccgcttcttggcca

SEQ ID NO: 244 - DNA, 20 bp, synthetic construct
  misc_feature 1..20: note = Synthetic
  source 1..20: mol_type = other DNA
ggtcggcccgcttcttggcc

SEQ ID NO: 245 - DNA, 20 bp, synthetic construct
  misc_feature 1..20: note = Synthetic
  source 1..20: mol_type = other DNA
aggtcggcccgcttcttggc

SEQ ID NO: 246 - DNA, 20 bp, synthetic construct
  misc_feature 1..20: note = Synthetic
  source 1..20: mol_type = other DNA
caggtcggcccgcttcttgg

SEQ ID NO: 247 - DNA, 20 bp, synthetic construct
  misc_feature 1..20: note = Synthetic
  source 1..20: mol_type = other DNA
ccaggtcggcccgcttcttg

SEQ ID NO: 248 - DNA, 20 bp, synthetic construct
  misc_feature 1..20: note = Synthetic
  source 1..20: mol_type = other DNA
accaggtcggcccgcttctt

SEQ ID NO: 249 - DNA, 20 bp, synthetic construct
  misc_feature 1..20: note = Synthetic
  source 1..20: mol_type = other DNA
caccaggtcggcccgcttct

SEQ ID NO: 250 - DNA, 20 bp, synthetic construct
  misc_feature 1..20: note = Synthetic
  source 1..20: mol_type = other DNA
ccaccaggtcggcccgcttc

SEQ ID NO: 251 - DNA, 20 bp, synthetic construct
  misc_feature 1..20: note = Synthetic
  source 1..20: mol_type = other DNA
tccaccaggtcggcccgctt

SEQ ID NO: 252 - DNA, 20 bp, synthetic construct
  misc_feature 1..20: note = Synthetic
  source 1..20: mol_type = other DNA
ctccaccaggtcggcccgct

SEQ ID NO: 253 - DNA, 20 bp, synthetic construct
  misc_feature 1..20: note = Synthetic
  source 1..20: mol_type = other DNA
tctccaccaggtcggcccgc

SEQ ID NO: 254 - DNA, 20 bp, synthetic construct
  misc_feature 1..20: note = Synthetic
  source 1..20: mol_type = other DNA
ttctccaccaggtcggcccg

SEQ ID NO: 255 - DNA, 20 bp, synthetic construct
  misc_feature 1..20: note = Synthetic
  source 1..20: mol_type = other DNA
cttctccaccaggtcggccc

SEQ ID NO: 256 - DNA, 20 bp, synthetic construct
  misc_feature 1..20: note = Synthetic
  source 1..20: mol_type = other DNA
accttctccaccaggtcggc

SEQ ID NO: 257 - DNA, 20 bp, synthetic construct
  misc_feature 1..20: note = Synthetic
  source 1..20: mol_type = other DNA
caccttctccaccaggtcgg

SEQ ID NO: 258 - DNA, 20 bp, synthetic construct
  misc_feature 1..20: note = Synthetic
  source 1..20: mol_type = other DNA
gcaccttctccaccaggtcg

SEQ ID NO: 259 - DNA, 20 bp, synthetic construct
  misc_feature 1..20: note = Synthetic
  source 1..20: mol_type = other DNA
ccgcaccttctccaccaggt

SEQ ID NO: 260 - DNA, 20 bp, synthetic construct
  misc_feature 1..20: note = Synthetic
  source 1..20: mol_type = other DNA
gccgcaccttctccaccagg

SEQ ID NO: 261 - DNA, 20 bp, synthetic construct
  misc_feature 1..20: note = Synthetic
  source 1..20: mol_type = other DNA
cgccgcaccttctccaccag

SEQ ID NO: 262 - DNA, 20 bp, synthetic construct
  misc_feature 1..20: note = Synthetic
  source 1..20: mol_type = other DNA
cgcgccgcaccttctccacc

SEQ ID NO: 263 - DNA, 20 bp, synthetic construct
  misc_feature 1..20: note = Synthetic
  source 1..20: mol_type = other DNA
tcgcgccgcaccttctccac

SEQ ID NO: 264 - DNA, 20 bp, synthetic construct
  misc_feature 1..20: note = Synthetic
  source 1..20: mol_type = other DNA
ctcgcgccgcaccttctcca

SEQ ID NO: 265 - DNA, 20 bp, synthetic construct
  misc_feature 1..20: note = Synthetic
  source 1..20: mol_type = other DNA
cctcgcgccgcaccttctcc

SEQ ID NO: 266 - DNA, 20 bp, synthetic construct
  misc_feature 1..20: note = Synthetic
  source 1..20: mol_type = other DNA
gcctcgcgccgcaccttctc

SEQ ID NO: 267 - DNA, 20 bp, synthetic construct
  misc_feature 1..20: note = Synthetic
  source 1..20: mol_type = other DNA
ggcctcgcgccgcaccttct

SEQ ID NO: 268 - DNA, 20 bp, synthetic construct
  misc_feature 1..20: note = Synthetic
  source 1..20: mol_type = other DNA
cggcctcgcgccgcaccttc

SEQ ID NO: 269 - DNA, 20 bp, synthetic construct
  misc_feature 1..20: note = Synthetic
  source 1..20: mol_type = other DNA
tcggcctcgcgccgcacctt

SEQ ID NO: 270 - DNA, 20 bp, synthetic construct
  misc_feature 1..20: note = Synthetic
  source 1..20: mol_type = other DNA
ctcggcctcgcgccgcacct

SEQ ID NO: 271 - DNA, 20 bp, synthetic construct
  misc_feature 1..20: note = Synthetic
  source 1..20: mol_type = other DNA
gctcggcctcgcgccgcacc

SEQ ID NO: 272 - DNA, 20 bp, synthetic construct
  misc_feature 1..20: note = Synthetic
  source 1..20: mol_type = other DNA
tgctcggcctcgcgccgcac

SEQ ID NO: 273 - DNA, 20 bp, synthetic construct
  misc_feature 1..20: note = Synthetic
  source 1..20: mol_type = other DNA
gcgctccttttcttcgcgcg

SEQ ID NO: 274 - DNA, 20 bp, synthetic construct
  misc_feature 1..20: note = Synthetic
  source 1..20: mol_type = other DNA
cgcgctccttttcttcgcgc

SEQ ID NO: 275 - DNA, 20 bp, synthetic construct
  misc_feature 1..20: note = Synthetic
  source 1..20: mol_type = other DNA
tcgcgctccttttcttcgcg

SEQ ID NO: 276 - DNA, 20 bp, synthetic construct
  misc_feature 1..20: note = Synthetic
  source 1..20: mol_type = other DNA
ctcgcgctccttttcttcgc

SEQ ID NO: 277 - DNA, 20 bp, synthetic construct
  misc_feature 1..20: note = Synthetic
  source 1..20: mol_type = other DNA
gctcgcgctccttttcttcg

SEQ ID NO: 278 - DNA, 20 bp, synthetic construct
  misc_feature 1..20: note = Synthetic
  source 1..20: mol_type = other DNA
cgctcgcgctccttttcttc

SEQ ID NO: 279 - DNA, 20 bp, synthetic construct
  misc_feature 1..20: note = Synthetic
  source 1..20: mol_type = other DNA
gcgctcgcgctccttttctt

SEQ ID NO: 280 - DNA, 20 bp, synthetic construct
  misc_feature 1..20: note = Synthetic
  source 1..20: mol_type = other DNA
cgcgctcgcgctccttttct

SEQ ID NO: 281 - DNA, 20 bp, synthetic construct
  misc_feature 1..20: note = Synthetic
  source 1..20: mol_type = other DNA
tcgcgctcgcgctccttttc

SEQ ID NO: 282 - DNA, 20 bp, synthetic construct
  misc_feature 1..20: note = Synthetic
  source 1..20: mol_type = other DNA
ctcgcgctcgcgctcctttt

SEQ ID NO: 283 - DNA, 20 bp, synthetic construct
  misc_feature 1..20: note = Synthetic
  source 1..20: mol_type = other DNA
gctcgcgctcgcgctccttt

SEQ ID NO: 284 - DNA, 20 bp, synthetic construct
  misc_feature 1..20: note = Synthetic
  source 1..20: mol_type = other DNA
cgctcgcgctcgcgctcctt

SEQ ID NO: 285 - DNA, 20 bp, synthetic construct
  misc_feature 1..20: note = Synthetic
  source 1..20: mol_type = other DNA
ccgctcgcgctcgcgctcct

SEQ ID NO: 286 - DNA, 20 bp, synthetic construct
  misc_feature 1..20: note = Synthetic
  source 1..20: mol_type = other DNA
cccgctcgcgctcgcgctcc

SEQ ID NO: 287 - DNA, 20 bp, synthetic construct
  misc_feature 1..20: note = Synthetic
  source 1..20: mol_type = other DNA
tcccgctcgcgctcgcgctc

SEQ ID NO: 288 - DNA, 20 bp, synthetic construct
  misc_feature 1..20: note = Synthetic
  source 1..20: mol_type = other DNA
ttcccgctcgcgctcgcgct

SEQ ID NO: 289 - DNA, 20 bp, synthetic construct
  misc_feature 1..20: note = Synthetic
  source 1..20: mol_type = other DNA
gttcccgctcgcgctcgcgc

SEQ ID NO: 290 - DNA, 20 bp, synthetic construct
  misc_feature 1..20: note = Synthetic
  source 1..20: mol_type = other DNA
cgttcccgctcgcgctcgcg

SEQ ID NO: 291 - DNA, 20 bp, synthetic construct
  misc_feature 1..20: note = Synthetic
  source 1..20: mol_type = other DNA
gcgttcccgctcgcgctcgc

SEQ ID NO: 292 - DNA, 20 bp, synthetic construct
  misc_feature 1..20: note = Synthetic
  source 1..20: mol_type = other DNA
cgcgttcccgctcgcgctcg

SEQ ID NO: 293 - DNA, 20 bp, synthetic construct
  misc_feature 1..20: note = Synthetic
  source 1..20: mol_type = other DNA
tcgcgttcccgctcgcgctc

SEQ ID NO: 294 - DNA, 20 bp, synthetic construct
  misc_feature 1..20: note = Synthetic
  source 1..20: mol_type = other DNA
ctcgcgttcccgctcgcgct

SEQ ID NO: 295 - DNA, 20 bp, synthetic construct
  misc_feature 1..20: note = Synthetic
  source 1..20: mol_type = other DNA
tctcgcgttcccgctcgcgc

SEQ ID NO: 296 - DNA, 20 bp, synthetic construct
  misc_feature 1..20: note = Synthetic
  source 1..20: mol_type = other DNA
ttctcgcgttcccgctcgcg

SEQ ID NO: 297 - DNA, 20 bp, synthetic construct
  misc_feature 1..20: note = Synthetic
  source 1..20: mol_type = other DNA
tttctcgcgttcccgctcgc

SEQ ID NO: 298 - DNA, 20 bp, synthetic construct
  misc_feature 1..20: note = Synthetic
  source 1..20: mol_type = other DNA
ctttctcgcgttcccgctcg

SEQ ID NO: 299 - DNA, 20 bp, synthetic construct
  misc_feature 1..20: note = Synthetic
  source 1..20: mol_type = other DNA
ctcgcgctccttctcgcgct

SEQ ID NO: 300 - DNA, 20 bp, synthetic construct
  misc_feature 1..20: note = Synthetic
  source 1..20: mol_type = other DNA
gctcgcgctccttctcgcgc

SEQ ID NO: 301 - DNA, 20 bp, synthetic construct
  misc_feature 1..20: note = Synthetic
  source 1..20: mol_type = other DNA
aagctcgcgctccttctcgc

SEQ ID NO: 302 - DNA, 20 bp, synthetic construct
  misc_feature 1..20: note = Synthetic
  source 1..20: mol_type = other DNA
caagctcgcgctccttctcg

SEQ ID NO: 303 - DNA, 20 bp, synthetic construct
  misc_feature 1..20: note = Synthetic
  source 1..20: mol_type = other DNA
ttcaagctcgcgctccttct

SEQ ID NO: 304 - DNA, 20 bp, synthetic construct
  misc_feature 1..20: note = Synthetic
  source 1..20: mol_type = other DNA
gttcaagctcgcgctccttc

SEQ ID NO: 305 - DNA, 20 bp, synthetic construct
  misc_feature 1..20: note = Synthetic
  source 1..20: mol_type = other DNA
cgttcaagctcgcgctcctt

SEQ ID NO: 306 - DNA, 20 bp, synthetic construct
  misc_feature 1..20: note = Synthetic
  source 1..20: mol_type = other DNA
gcgttcaagctcgcgctcct

SEQ ID NO: 307 - DNA, 20 bp, synthetic construct
  misc_feature 1..20: note = Synthetic
  source 1..20: mol_type = other DNA
ccgcactgcccggttcaaat

SEQ ID NO: 308 - DNA, 20 bp, synthetic construct
  misc_feature 1..20: note = Synthetic
  source 1..20: mol_type = other DNA
accgcactgcccggttcaaa

SEQ ID NO: 309 - DNA, 20 bp, synthetic construct
  misc_feature 1..20: note = Synthetic
  source 1..20: mol_type = other DNA
ccaccgcactgcccggttca

SEQ ID NO: 310 - DNA, 20 bp, synthetic construct
  misc_feature 1..20: note = Synthetic
  source 1..20: mol_type = other DNA
gccaccgcactgcccggttc

SEQ ID NO: 311 - DNA, 20 bp, synthetic construct
  misc_feature 1..20: note = Synthetic
  source 1..20: mol_type = other DNA
tagccaccgcactgcccggt

SEQ ID NO: 312 - DNA, 20 bp, synthetic construct
  misc_feature 1..20: note = Synthetic
  source 1..20: mol_type = other DNA
gtagccaccgcactgcccgg

SEQ ID NO: 313 - DNA, 20 bp, synthetic construct
  misc_feature 1..20: note = Synthetic
  source 1..20: mol_type = other DNA
ctgtagccaccgcactgccc

SEQ ID NO: 314 - DNA, 20 bp, synthetic construct
  misc_feature 1..20: note = Synthetic
  source 1..20: mol_type = other DNA
actgtagccaccgcactgcc

SEQ ID NO: 315 - DNA, 20 bp, synthetic construct
  misc_feature 1..20: note = Synthetic
  source 1..20: mol_type = other DNA
cccgggtccactgcccccag

SEQ ID NO: 316 - DNA, 20 bp, synthetic construct
  misc_feature 1..20: note = Synthetic
  source 1..20: mol_type = other DNA
gtgctgcctctcagctgcca

SEQ ID NO: 317 - DNA, 20 bp, synthetic construct
  misc_feature 1..20: note = Synthetic
  source 1..20: mol_type = other DNA
cgtgctgcctctcagctgcc

SEQ ID NO: 318 - DNA, 20 bp, synthetic construct
  misc_feature 1..20: note = Synthetic
  source 1..20: mol_type = other DNA
gcgtgctgcctctcagctgc

SEQ ID NO: 319 - DNA, 20 bp, synthetic construct
  misc_feature 1..20: note = Synthetic
  source 1..20: mol_type = other DNA
ctgcgtgctgcctctcagct

SEQ ID NO: 320 - DNA, 20 bp, synthetic construct
  misc_feature 1..20: note = Synthetic
  source 1..20: mol_type = other DNA
tctgcgtgctgcctctcagc

SEQ ID NO: 321 - DNA, 20 bp, synthetic construct
  misc_feature 1..20: note = Synthetic
  source 1..20: mol_type = other DNA
ttctgcgtgctgcctctcag

SEQ ID NO: 322 - DNA, 20 bp, synthetic construct
  misc_feature 1..20: note = Synthetic
  source 1..20: mol_type = other DNA
tttctgcgtgctgcctctca

SEQ ID NO: 323 - DNA, 20 bp, synthetic construct
  misc_feature 1..20: note = Synthetic
  source 1..20: mol_type = other DNA
ctttctgcgtgctgcctctc

SEQ ID NO: 324 - DNA, 20 bp, synthetic construct
  misc_feature 1..20: note = Synthetic
  source 1..20: mol_type = other DNA
cctttctgcgtgctgcctct

SEQ ID NO: 325 - DNA, 20 bp, synthetic construct
  misc_feature 1..20: note = Synthetic
  source 1..20: mol_type = other DNA
ccctttctgcgtgctgcctc

SEQ ID NO: 326 - DNA, 20 bp, synthetic construct
  misc_feature 1..20: note = Synthetic
  source 1..20: mol_type = other DNA
accctttctgcgtgctgcct

SEQ ID NO: 327 - DNA, 20 bp, synthetic construct
  misc_feature 1..20: note = Synthetic
  source 1..20: mol_type = other DNA
caccctttctgcgtgctgcc

SEQ ID NO: 328 - DNA, 20 bp, synthetic construct
  misc_feature 1..20: note = Synthetic
  source 1..20: mol_type = other DNA
ccaccctttctgcgtgctgc

SEQ ID NO: 329 - DNA, 20 bp, synthetic construct
  misc_feature 1..20: note = Synthetic
  source 1..20: mol_type = other DNA
gccaccctttctgcgtgctg

SEQ ID NO: 330 - DNA, 20 bp, synthetic construct
  misc_feature 1..20: note = Synthetic
  source 1..20: mol_type = other DNA
cgccaccctttctgcgtgct

SEQ ID NO: 331 - DNA, 20 bp, synthetic construct
  misc_feature 1..20: note = Synthetic
  source 1..20: mol_type = other DNA
ccgccaccctttctgcgtgc

SEQ ID NO: 332 - DNA, 20 bp, synthetic construct
  misc_feature 1..20: note = Synthetic
  source 1..20: mol_type = other DNA
gccgccaccctttctgcgtg

SEQ ID NO: 333 - DNA, 20 bp, synthetic construct
  misc_feature 1..20: note = Synthetic
  source 1..20: mol_type = other DNA
ggccgccaccctttctgcgt

SEQ ID NO: 334 - DNA, 20 bp, synthetic construct
  misc_feature 1..20: note = Synthetic
  source 1..20: mol_type = other DNA
gggccgccaccctttctgcg

SEQ ID NO: 335 - DNA, 20 bp, synthetic construct
  misc_feature 1..20: note = Synthetic
  source 1..20: mol_type = other DNA
agggccgccaccctttctgc

SEQ ID NO: 336 - DNA, 20 bp, synthetic construct
  misc_feature 1..20: note = Synthetic
  source 1..20: mol_type = other DNA
cagggccgccaccctttctg

SEQ ID NO: 337 - DNA, 20 bp, synthetic construct
  misc_feature 1..20: note = Synthetic
  source 1..20: mol_type = other DNA
ggcagaaagggaggccggca

SEQ ID NO: 338 - DNA, 20 bp, synthetic construct
  misc_feature 1..20: note = Synthetic
  source 1..20: mol_type = other DNA
gggcagaaagggaggccggc

SEQ ID NO: 339 - DNA, 20 bp, synthetic construct
  misc_feature 1..20: note = Synthetic
  source 1..20: mol_type = other DNA
ggggcagaaagggaggccgg

SEQ ID NO: 340 - DNA, 20 bp, synthetic construct
  misc_feature 1..20: note = Synthetic
  source 1..20: mol_type = other DNA
cggggcagaaagggaggccg

SEQ ID NO: 341 - DNA, 20 bp, synthetic construct
  misc_feature 1..20: note = Synthetic
  source 1..20: mol_type = other DNA
tcggggcagaaagggaggcc

SEQ ID NO: 342 - DNA, 20 bp, synthetic construct
  misc_feature 1..20: note = Synthetic
  source 1..20: mol_type = other DNA
atcggggcagaaagggaggc

SEQ ID NO: 343 - DNA, 20 bp, synthetic construct
  misc_feature 1..20: note = Synthetic
  source 1..20: mol_type = other DNA
catcggggcagaaagggagg

SEQ ID NO: 344 - DNA, 20 bp, synthetic construct
  misc_feature 1..20: note = Synthetic
  source 1..20: mol_type = other DNA
acatcggggcagaaagggag

SEQ ID NO: 345 - DNA, 20 bp, synthetic construct
  misc_feature 1..20: note = Synthetic
  source 1..20: mol_type = other DNA
gacatcggggcagaaaggga

SEQ ID NO: 346 - DNA, 20 bp, synthetic construct
  misc_feature 1..20: note = Synthetic
  source 1..20: mol_type = other DNA
tgacatcggggcagaaaggg

SEQ ID NO: 347 - DNA, 20 bp, synthetic construct
  misc_feature 1..20: note = Synthetic
  source 1..20: mol_type = other DNA
ctgacatcggggcagaaagg

SEQ ID NO: 348 - DNA, 20 bp, synthetic construct
  misc_feature 1..20: note = Synthetic
  source 1..20: mol_type = other DNA
gctgacatcggggcagaaag

SEQ ID NO: 349 - DNA, 20 bp, synthetic construct
  misc_feature 1..20: note = Synthetic
  source 1..20: mol_type = other DNA
tgctgacatcggggcagaaa

SEQ ID NO: 350 - DNA, 20 bp, synthetic construct
  misc_feature 1..20: note = Synthetic
  source 1..20: mol_type = other DNA
gctgctgacatcggggcaga

SEQ ID NO: 351 - DNA, 20 bp, synthetic construct
  misc_feature 1..20: note = Synthetic
  source 1..20: mol_type = other DNA
agctgctgacatcggggcag

SEQ ID NO: 352 - DNA, 20 bp, synthetic construct
  misc_feature 1..20: note = Synthetic
  source 1..20: mol_type = other DNA
gagctgctgacatcggggca

SEQ ID NO: 353 - DNA, 20 bp, synthetic construct
  misc_feature 1..20: note = Synthetic
  source 1..20: mol_type = other DNA
atgagctgctgacatcgggg

SEQ ID NO: 354 - DNA, 20 bp, synthetic construct
  misc_feature 1..20: note = Synthetic
  source 1..20: mol_type = other DNA
gatgagctgctgacatcggg

SEQ ID NO: 355 - DNA, 20 bp, synthetic construct
  misc_feature 1..20: note = Synthetic
  source 1..20: mol_type = other DNA
tgatgagctgctgacatcgg

SEQ ID NO: 356 - DNA, 20 bp, synthetic construct
  misc_feature 1..20: note = Synthetic
  source 1..20: mol_type = other DNA
gctgatgagctgctgacatc

SEQ ID NO: 357 - DNA, 20 bp, synthetic construct
  misc_feature 1..20: note = Synthetic
  source 1..20: mol_type = other DNA
agctgatgagctgctgacat

SEQ ID NO: 358 - DNA, 20 bp, synthetic construct
  misc_feature 1..20: note = Synthetic
  source 1..20: mol_type = other DNA
cagctgatgagctgctgaca

SEQ ID NO: 359 - DNA, 20 bp, synthetic construct
  misc_feature 1..20: note = Synthetic
  source 1..20: mol_type = other DNA
gcagctgatgagctgctgac

SEQ ID NO: 360 - DNA, 20 bp, synthetic construct
  misc_feature 1..20: note = Synthetic
  source 1..20: mol_type = other DNA
tgcagctgatgagctgctga

SEQ ID NO: 361 - DNA, 20 bp, synthetic construct
  misc_feature 1..20: note = Synthetic
  source 1..20: mol_type = other DNA
ctgcagctgatgagctgctg

SEQ ID NO: 362 - DNA, 20 bp, synthetic construct
  misc_feature 1..20: note = Synthetic
  source 1..20: mol_type = other DNA
cctgcagctgatgagctgct

SEQ ID NO: 363 - DNA, 20 bp, synthetic construct
  misc_feature 1..20: note = Synthetic
  source 1..20: mol_type = other DNA
gcctgcagctgatgagctgc

SEQ ID NO: 364 - DNA, 20 bp, synthetic construct
  misc_feature 1..20: note = Synthetic
  source 1..20: mol_type = other DNA
ggcctgcagctgatgagctg

SEQ ID NO: 365 - DNA, 20 bp, synthetic construct
  misc_feature 1..20: note = Synthetic
  source 1..20: mol_type = other DNA
tggcctgcagctgatgagct

SEQ ID NO: 366 - DNA, 20 bp, synthetic construct
  misc_feature 1..20: note = Synthetic
  source 1..20: mol_type = other DNA
atggcctgcagctgatgagc

SEQ ID NO: 367 - DNA, 20 bp, synthetic construct
  misc_feature 1..20: note = Synthetic
  source 1..20: mol_type = other DNA
catggcctgcagctgatgag

SEQ ID NO: 368 - DNA, 20 bp, synthetic construct
  misc_feature 1..20: note = Synthetic
  source 1..20: mol_type = other DNA
gcatggcctgcagctgatga

SEQ ID NO: 369 - DNA, 20 bp, synthetic construct
  misc_feature 1..20: note = Synthetic
  source 1..20: mol_type = other DNA
tgcatggcctgcagctgatg

SEQ ID NO: 370 - DNA, 20 bp, synthetic construct
  misc_feature 1..20: note = Synthetic
  source 1..20: mol_type = other DNA
cagctcagctgactgtgcgt

SEQ ID NO: 371 - DNA, 20 bp, synthetic construct
  misc_feature 1..20: note = Synthetic
  source 1..20: mol_type = other DNA
gcagctcagctgactgtgcg

SEQ ID NO: 372 - DNA, 20 bp, synthetic construct
  misc_feature 1..20: note = Synthetic
  source 1..20: mol_type = other DNA
tgcagctcagctgactgtgc

SEQ ID NO: 373 - DNA, 20 bp, synthetic construct
  misc_feature 1..20: note = Synthetic
  source 1..20: mol_type = other DNA
ctgcagctcagctgactgtg

SEQ ID NO: 374 - DNA, 20 bp, synthetic construct
  misc_feature 1..20: note = Synthetic
  source 1..20: mol_type = other DNA
gctgcagctcagctgactgt

SEQ ID NO: 375 - DNA, 20 bp, synthetic construct
  misc_feature 1..20: note = Synthetic
  source 1..20: mol_type = other DNA
cgctgcagctcagctgactg

SEQ ID NO: 376 - DNA, 20 bp, synthetic construct
  misc_feature 1..20: note = Synthetic
  source 1..20: mol_type = other DNA
gcgctgcagctcagctgact

SEQ ID NO: 377 - DNA, 20 bp, synthetic construct
  misc_feature 1..20: note = Synthetic
  source 1..20: mol_type = other DNA
agcgctgcagctcagctgac

SEQ ID NO: 378 - DNA, 20 bp, synthetic construct
  misc_feature 1..20: note = Synthetic
  source 1..20: mol_type = other DNA
aagcgctgcagctcagctga

SEQ ID NO: 379 - DNA, 20 bp, synthetic construct
  misc_feature 1..20: note = Synthetic
  source 1..20: mol_type = other DNA
caagcgctgcagctcagctg

SEQ ID NO: 380 - DNA, 20 bp, synthetic construct
  misc_feature 1..20: note = Synthetic
  source 1..20: mol_type = other DNA
ccaagcgctgcagctcagct

SEQ ID NO: 381 - DNA, 20 bp, synthetic construct
  misc_feature 1..20: note = Synthetic
  source 1..20: mol_type = other DNA
gccaagcgctgcagctcagc

SEQ ID NO: 382 - DNA, 20 bp, synthetic construct
  misc_feature 1..20: note = Synthetic
  source 1..20: mol_type = other DNA
cgccaagcgctgcagctcag

SEQ ID NO: 383 - DNA, 20 bp, synthetic construct
  misc_feature 1..20: note = Synthetic
  source 1..20: mol_type = other DNA
gcgccaagcgctgcagctca

SEQ ID NO: 384 - DNA, 20 bp, synthetic construct
  misc_feature 1..20: note = Synthetic
  source 1..20: mol_type = other DNA
agcgccaagcgctgcagctc

SEQ ID NO: 385 - DNA, 20 bp, synthetic construct
  misc_feature 1..20: note = Synthetic
  source 1..20: mol_type = other DNA
ccagcgccaagcgctgcagc

SEQ ID NO: 386 - DNA, 20 bp, synthetic construct
  misc_feature 1..20: note = Synthetic
  source 1..20: mol_type = other DNA
tccagcgccaagcgctgcag

SEQ ID NO: 387 - DNA, 20 bp, synthetic construct
  misc_feature 1..20: note = Synthetic
  source 1..20: mol_type = other DNA
ttccagcgccaagcgctgca

SEQ ID NO: 388 - DNA, 20 bp, synthetic construct
  misc_feature 1..20: note = Synthetic
  source 1..20: mol_type = other DNA
tgttccagcgccaagcgctg

SEQ ID NO: 389 - DNA, 20 bp, synthetic construct
  misc_feature 1..20: note = Synthetic
  source 1..20: mol_type = other DNA
ctgttccagcgccaagcgct

SEQ ID NO: 390 - DNA, 20 bp, synthetic construct
  misc_feature 1..20: note = Synthetic
  source 1..20: mol_type = other DNA
gctgttccagcgccaagcgc

SEQ ID NO: 391 - DNA, 20 bp, synthetic construct
  misc_feature 1..20: note = Synthetic
  source 1..20: mol_type = other DNA
ctgctgttccagcgccaagc

SEQ ID NO: 392 - DNA, 20 bp, synthetic construct
  misc_feature 1..20: note = Synthetic
  source 1..20: mol_type = other DNA
gctgctgttccagcgccaag

SEQ ID NO: 393 - DNA, 20 bp, synthetic construct
  misc_feature 1..20: note = Synthetic
  source 1..20: mol_type = other DNA
tgctgctgttccagcgccaa

SEQ ID NO: 394 - DNA, 20 bp, synthetic construct
  misc_feature 1..20: note = Synthetic
  source 1..20: mol_type = other DNA
ctgctgctgttccagcgcca

SEQ ID NO: 395 - DNA, 20 bp, synthetic construct
  misc_feature 1..20: note = Synthetic
  source 1..20: mol_type = other DNA
actgctgctgttccagcgcc

SEQ ID NO: 396 - DNA, 20 bp, synthetic construct
  misc_feature 1..20: note = Synthetic
  source 1..20: mol_type = other DNA
cactgctgctgttccagcgc

SEQ ID NO: 397 - DNA, 20 bp, synthetic construct
  misc_feature 1..20: note = Synthetic
  source 1..20: mol_type = other DNA
ccactgctgctgttccagcg

SEQ ID NO: 398 - DNA, 20 bp, synthetic construct
  misc_feature 1..20: note = Synthetic
  source 1..20: mol_type = other DNA
gccactgctgctgttccagc

SEQ ID NO: 399 - DNA, 20 bp, synthetic construct
  misc_feature 1..20: note = Synthetic
  source 1..20: mol_type = other DNA
agccactgctgctgttccag

SEQ ID NO: 400 - DNA, 20 bp, synthetic construct
  misc_feature 1..20: note = Synthetic
  source 1..20: mol_type = other DNA
cagccactgctgctgttcca

SEQ ID NO: 401 - DNA, 20 bp, synthetic construct
  misc_feature 1..20: note = Synthetic
  source 1..20: mol_type = other DNA
gcagccactgctgctgttcc

SEQ ID NO: 402 - DNA, 20 bp, synthetic construct
  misc_feature 1..20: note = Synthetic
  source 1..20: mol_type = other DNA
tgcagccactgctgctgttc

SEQ ID NO: 403 - DNA, 20 bp, synthetic construct
  misc_feature 1..20: note = Synthetic
  source 1..20: mol_type = other DNA
atgcagccactgctgctgtt

SEQ ID NO: 404 - DNA, 20 bp, synthetic construct
  misc_feature 1..20: note = Synthetic
  source 1..20: mol_type = other DNA
ggcagcggcacactgtgcag

SEQ ID NO: 405 - DNA, 20 bp, synthetic construct
  misc_feature 1..20: note = Synthetic
  source 1..20: mol_type = other DNA
aggcagcggcacactgtgca

SEQ ID NO: 406 - DNA, 20 bp, synthetic construct
  misc_feature 1..20: note = Synthetic
  source 1..20: mol_type = other DNA
caggcagcggcacactgtgc

SEQ ID NO: 407 - DNA, 20 bp, synthetic construct
  misc_feature 1..20: note = Synthetic
  source 1..20: mol_type = other DNA
gcaggcagcggcacactgtg

SEQ ID NO: 408 - DNA, 20 bp, synthetic construct
  misc_feature 1..20: note = Synthetic
  source 1..20: mol_type = other DNA
ggcaggcagcggcacactgt

SEQ ID NO: 409 - DNA, 20 bp, synthetic construct
  misc_feature 1..20: note = Synthetic
  source 1..20: mol_type = other DNA
ttggccttctgtctgtccct

SEQ ID NO: 410 - DNA, 20 bp, synthetic construct
  misc_feature 1..20: note = Synthetic
  source 1..20: mol_type = other DNA
cttggccttctgtctgtccc

SEQ ID NO: 411 - DNA, 20 bp, synthetic construct
  misc_feature 1..20: note = Synthetic
  source 1..20: mol_type = other DNA
ccttggccttctgtctgtcc

SEQ ID NO: 412 - DNA, 20 bp, synthetic construct
  misc_feature 1..20: note = Synthetic
  source 1..20: mol_type = other DNA
gccttggccttctgtctgtc

SEQ ID NO: 413 - DNA, 20 bp, synthetic construct
  misc_feature 1..20: note = Synthetic
  source 1..20: mol_type = other DNA
ggccttggccttctgtctgt

SEQ ID NO: 414 - DNA, 20 bp, synthetic construct
  misc_feature 1..20: note = Synthetic
  source 1..20: mol_type = other DNA
gggccttggccttctgtctg

SEQ ID NO: 415 - DNA, 20 bp, synthetic construct
  misc_feature 1..20: note = Synthetic
  source 1..20: mol_type = other DNA
cgggccttggccttctgtct

SEQ ID NO: 416 - DNA, 20 bp, synthetic construct
  misc_feature 1..20: note = Synthetic
  source 1..20: mol_type = other DNA
tcgggccttggccttctgtc

SEQ ID NO: 417 - DNA, 20 bp, synthetic construct
  misc_feature 1..20: note = Synthetic
  source 1..20: mol_type = other DNA
atcgggccttggccttctgt

SEQ ID NO: 418 - DNA, 20 bp, synthetic construct
  misc_feature 1..20: note = Synthetic
  source 1..20: mol_type = other DNA
catcgggccttggccttctg

SEQ ID NO: 419 - DNA, 20 bp, synthetic construct
  misc_feature 1..20: note = Synthetic
  source 1..20: mol_type = other DNA
acatcgggccttggccttct

SEQ ID NO: 420 - DNA, 20 bp, synthetic construct
  misc_feature 1..20: note = Synthetic
  source 1..20: mol_type = other DNA
cacatcgggccttggccttc

SEQ ID NO: 421 - DNA, 20 bp, synthetic construct
  misc_feature 1..20: note = Synthetic
  source 1..20: mol_type = other DNA
ccacatcgggccttggcctt

SEQ ID NO: 422 - DNA, 20 bp, synthetic construct
  misc_feature 1..20: note = Synthetic
  source 1..20: mol_type = other DNA
accacatcgggccttggcct

SEQ ID NO: 423 - DNA, 20 bp, synthetic construct
  misc_feature 1..20: note = Synthetic
  source 1..20: mol_type = other DNA
caccacatcgggccttggcc

SEQ ID NO: 424 - DNA, 20 bp, synthetic construct
  misc_feature 1..20: note = Synthetic
  source 1..20: mol_type = other DNA
cacaccacatcgggccttgg

SEQ ID NO: 425 - DNA, 20 bp, synthetic construct
  misc_feature 1..20: note = Synthetic
  source 1..20: mol_type = other DNA
gcacaccacatcgggccttg

SEQ ID NO: 426 - DNA, 20 bp, synthetic construct
  misc_feature 1..20: note = Synthetic
  source 1..20: mol_type = other DNA
tgcacaccacatcgggcctt

SEQ ID NO: 427 - DNA, 20 bp, synthetic construct
  misc_feature 1..20: note = Synthetic
  source 1..20: mol_type = other DNA
tctgcacaccacatcgggcc

SEQ ID NO: 428 - DNA, 20 bp, synthetic construct
  misc_feature 1..20: note = Synthetic
  source 1..20: mol_type = other DNA
ctctgcacaccacatcgggc

SEQ ID NO: 429 - DNA, 20 bp, synthetic construct
  misc_feature 1..20: note = Synthetic
  source 1..20: mol_type = other DNA
cctctgcacaccacatcggg

SEQ ID NO: 430 - DNA, 20 bp, synthetic construct
  misc_feature 1..20: note = Synthetic
  source 1..20: mol_type = other DNA
cacctctgcacaccacatcg

SEQ ID NO: 431 - DNA, 20 bp, synthetic construct
  misc_feature 1..20: note = Synthetic
  source 1..20: mol_type = other DNA
ccacctctgcacaccacatc

SEQ ID NO: 432 - DNA, 20 bp, synthetic construct
  misc_feature 1..20: note = Synthetic
  source 1..20: mol_type = other DNA
cccacctctgcacaccacat

SEQ ID NO: 433 - DNA, 20 bp, synthetic construct
  misc_feature 1..20: note = Synthetic
  source 1..20: mol_type = other DNA
ccccacctctgcacaccaca

SEQ ID NO: 434 - DNA, 20 bp, synthetic construct
  misc_feature 1..20: note = Synthetic
  source 1..20: mol_type = other DNA
tccccacctctgcacaccac

SEQ ID NO: 435 - DNA, 20 bp, synthetic construct
  misc_feature 1..20: note = Synthetic
  source 1..20: mol_type = other DNA
ctccccacctctgcacacca

SEQ ID NO: 436 - DNA, 20 bp, synthetic construct
  misc_feature 1..20: note = Synthetic
  source 1..20: mol_type = other DNA
cctccccacctctgcacacc

SEQ ID NO: 437 - DNA, 20 bp, synthetic construct
  misc_feature 1..20: note = Synthetic
  source 1..20: mol_type = other DNA
acctccccacctctgcacac

SEQ ID NO: 438 - DNA, 20 bp, synthetic construct
  misc_feature 1..20: note = Synthetic
  source 1..20: mol_type = other DNA
cacctccccacctctgcaca

SEQ ID NO: 439 - DNA, 20 bp, synthetic construct
  misc_feature 1..20: note = Synthetic
  source 1..20: mol_type = other DNA
ccacctccccacctctgcac

SEQ ID NO: 440 - DNA, 20 bp, synthetic construct
  misc_feature 1..20: note = Synthetic
  source 1..20: mol_type = other DNA
aggggcaggggtggcacacg

SEQ ID NO: 441 - DNA, 20 bp, synthetic construct
  misc_feature 1..20: note = Synthetic
  source 1..20: mol_type = other DNA
gaggggcaggggtggcacac

SEQ ID NO: 442 - DNA, 20 bp, synthetic construct
  misc_feature 1..20: note = Synthetic
  source 1..20: mol_type = other DNA
ggaggggcaggggtggcaca

SEQ ID NO: 443 - DNA, 20 bp, synthetic construct
  misc_feature 1..20: note = Synthetic
  source 1..20: mol_type = other DNA
gggaggggcaggggtggcac

SEQ ID NO: 444 - DNA, 20 bp, synthetic construct
  misc_feature 1..20: note = Synthetic
  source 1..20: mol_type = other DNA
ggggaggggcaggggtggca

SEQ ID NO: 445 - DNA, 20 bp, synthetic construct
  misc_feature 1..20: note = Synthetic
  source 1..20: mol_type = other DNA
cggggaggggcaggggtggc

SEQ ID NO: 446 - DNA, 20 bp, synthetic construct
  misc_feature 1..20: note = Synthetic
  source 1..20: mol_type = other DNA
tcggggaggggcaggggtgg

SEQ ID NO: 447 - DNA, 20 bp, synthetic construct
  misc_feature 1..20: note = Synthetic
  source 1..20: mol_type = other DNA
atcggggaggggcaggggtg

SEQ ID NO: 448 - DNA, 20 bp, synthetic construct
  misc_feature 1..20: note = Synthetic
  source 1..20: mol_type = other DNA
gatcggggaggggcaggggt

SEQ ID NO: 449 - DNA, 20 bp, synthetic construct
  misc_feature 1..20: note = Synthetic
  source 1..20: mol_type = other DNA
ggatcggggaggggcagggg

SEQ ID NO: 450 - DNA, 20 bp, synthetic construct
  misc_feature 1..20: note = Synthetic
  source 1..20: mol_type = other DNA
gggatcggggaggggcaggg

SEQ ID NO: 451 - DNA, 20 bp, synthetic construct
  misc_feature 1..20: note = Synthetic
  source 1..20: mol_type = other DNA
agggatcggggaggggcagg

SEQ ID NO: 452 - DNA, 20 bp, synthetic construct
  misc_feature 1..20: note = Synthetic
  source 1..20: mol_type = other DNA
cagggatcggggaggggcag

SEQ ID NO: 453 - DNA, 20 bp, synthetic construct
  misc_feature 1..20: note = Synthetic
  source 1..20: mol_type = other DNA
acagggatcggggaggggca

SEQ ID NO: 454 - DNA, 20 bp, synthetic construct
  misc_feature 1..20: note = Synthetic
  source 1..20: mol_type = other DNA
cacagggatcggggaggggc

SEQ ID NO: 455 - DNA, 20 bp, synthetic construct
  misc_feature 1..20: note = Synthetic
  source 1..20: mol_type = other DNA
acacagggatcggggagggg

SEQ ID NO: 456 - DNA, 20 bp, synthetic construct
  misc_feature 1..20: note = Synthetic
  source 1..20: mol_type = other DNA
cacacagggatcggggaggg

SEQ ID NO: 457 - DNA, 20 bp, synthetic construct
  misc_feature 1..20: note = Synthetic
  source 1..20: mol_type = other DNA
gcacacagggatcggggagg

SEQ ID NO: 458 - DNA, 20 bp, synthetic construct
  misc_feature 1..20: note = Synthetic
  source 1..20: mol_type = other DNA
cgcacacagggatcggggag

SEQ ID NO: 459 - DNA, 20 bp, synthetic construct
  misc_feature 1..20: note = Synthetic
  source 1..20: mol_type = other DNA
gcgcacacagggatcgggga

SEQ ID NO: 460 - DNA, 20 bp, synthetic construct
  misc_feature 1..20: note = Synthetic
  source 1..20: mol_type = other DNA
cgcgcacacagggatcgggg

SEQ ID NO: 461 - DNA, 20 bp, synthetic construct
  misc_feature 1..20: note = Synthetic
  source 1..20: mol_type = other DNA
gcgcgcacacagggatcggg

SEQ ID NO: 462 - DNA, 20 bp, synthetic construct
  misc_feature 1..20: note = Synthetic
  source 1..20: mol_type = other DNA
ggcgcgcacacagggatcgg

SEQ ID NO: 463 - DNA, 20 bp, synthetic construct
  misc_feature 1..20: note = Synthetic
  source 1..20: mol_type = other DNA
ggggcgcgcacacagggatc

SEQ ID NO: 464 - DNA, 20 bp, synthetic construct
  misc_feature 1..20: note = Synthetic
  source 1..20: mol_type = other DNA
gggggcgcgcacacagggat

SEQ ID NO: 465 - DNA, 20 bp, synthetic construct
  misc_feature 1..20: note = Synthetic
  source 1..20: mol_type = other DNA
tcaacaagcagggtcggagt

SEQ ID NO: 466 - DNA, 20 bp, synthetic construct
  misc_feature 1..20: note = Synthetic
  source 1..20: mol_type = other DNA
ttgaacgcagcgtgaagttg

SEQ ID NO: 467 - DNA, 21 bp, synthetic construct
  misc_feature 1..21: note = Synthetic
  source 1..21: mol_type = other DNA
cttcggttgtcctggtcgata

SEQ ID NO: 468 - DNA, 20 bp, synthetic construct
  misc_feature 1..20: note = Synthetic
  source 1..20: mol_type = other DNA
ttgcgattgccaggagacat

SEQ ID NO: 469 - DNA, 22 bp, synthetic construct
  misc_feature 1..22: note = Synthetic
  source 1..22: mol_type = other DNA
gaagatcaagatcattgctcct

SEQ ID NO: 470 - DNA, 20 bp, synthetic construct
  misc_feature 1..20: note = Synthetic
  source 1..20: mol_type = other DNA
tactcctgcttgctgatcca

SEQ ID NO: 471 - DNA, 4355 bp, Homo sapiens
  source 1..4355: mol_type = genomic DNA
gcaggacgccatactggacgccaagtgggaggaacttcaaggctgtcccctgcgggcctcccgctctgcttctgcgaaggtttcattgaaaacagatcctgcaaaagttccaggtgcccacactggaaacttggagatcctgcttcccagaccacagctgtggggaacttggggtggagcagagaagtttctgtattcagctgcccaggcagaggagaatggggtctccacagcctgaagaatgaagacacgacagaataaagactcgatgtcaatgaggagtggacggaagaaagaggcccctgggccccgggaagaactgagatcgaggggccgggcctcccctggaggggtcagcacgtccagcagtgatggcaaagctgagaagtccaggcagacagccaagaaggcccgagtagaggaagcctccaccccaaaggtcaacaagcagggtcggagtgaggagatctcagagagtgaaagtgaggagaccaatgcaccaaaaaagaccaaaactgagcaggaactccctcggccacagtctccctccgatctggatagcttggacgggcggagccttaatgatgatggcagcagcgaccctagggatatcgaccaggacaaccgaagcacgtcccccagtatctacagccctggaagtgtggagaatgactctgactcatcttctggcctgtcccagggcccagcccgcccctaccacccacctccactctttcctccttcccctcaaccgccagacagcacccctcgacagccagaggctagctttgaaccccatccttctgtgacacccactggatatcatgctcccatggagccccccacatctcgaatgttccaggctcctcctggggcccctccccctcacccacagctctatcctgggggcactggtggagttttgtctggacccccaatgggtcccaaggggggaggggctgcctcatcagtggggggccctaatgggggtaagcagcaccccccacccactactcccatttcagtatcaagctctggggctagtggtgctcccccaacaaagccgcctaccactccagtgggtggtgggaacctaccttctgctccaccaccagccaacttcccccatgtgacaccgaacctgcctcccccacctgccctgagacccctcaacaatgcatcagcctctccccctggcctgggggcccaaccactacctggtcatctgccctctccccacgccatgggacagggtatgggtggacttcctcctggcccagagaagggcccaactctggctccttcaccccactctctgcctcctgcttcctcttctgctccagcgccccccatgaggtttccttattcatcctctagtagtagctctgcagcagcctcctcttccagttcttcctcctcttcctctgcctcccccttcccagcttcccaggcattgcccagctacccccactctttccctcccccaacaagcctctctgtctccaatcagccccccaagtatactcagccttctctcccatcccaggctgtgtggagccagggtcccccaccacctcctccctatggccgcctcttagccaacagcaatgcccatccaggccccttccctccctctactggggcccagtccaccgcccacccaccagtctcaacacatcaccatcaccaccagcaacagcaacagcagcagcagcagcagcagcagcagcagcagcagcagcagcagcatcacggaaactctgggccccctcctcctggagcatttccccacccactggagggcggtagctcccaccacgcacacccttacgccatgtctccctccctggggtctctgaggccctacccaccagggccagcacacctgcccccacctcacagccaggtgtcctacagccaagcaggccccaatggccctccagtctcttcctcttccaactcttcctcttccacttctcaagggtcctacccatgttcacacccctccccttcccagggccctcaaggggcgccctaccctttcccaccggtgcctacggtcaccacctcttcggctaccctttccacggtcattgccaccgtggcttcctcgccagcaggctacaaaacggcctccccacctgggcccccaccgtacggaaagagagccccgtccccgggggcctacaagacagccaccccacccggatacaaacccgggtcgcctccctccttccgaacggggaccccaccgggctatcgaggaacctcgccacctgcaggcccagggaccttcaagccgggctcgcccaccgtgggacctgggcccctgccacctgcggggccctcaggcctgccatcgctgccaccaccacctgcggcccctgcctcagggccgcccctgagcgccacgcagatcaaacaggagccggctgaggagtatgagacccccgagagcccggtgcccccagcccgcagcccctcgccccctcccaaggtggtagatgtacccagccatgccagtcagtctgccaggttcaacaaacacctggatcgcggcttcaactcgtgcgcgcgcagcgacctgtacttcgtgccactggagggctccaagctggccaagaagcgggccgacctggtggagaaggtgcggcgcgaggccgagcagcgcgcgcgcgaagaaaaggagcgcgagcgcgagcgggaacgcgagaaagagcgcgagcgcgagaaggagcgcgagcttgaacgcagcgtgaagttggctcaggagggccgtgctccggtggaatgcccatctctgggcccagtgccccatcgccctccatttgaaccgggcagtgcggtggctacagtgcccccctacctgggtcctgacactccagccttgcgcactctcagtgaatatgcccggcctcatgtcatgtctcctggcaatcgcaaccatccattctacgtgcccctgggggcagtggacccggggctcctgggttacaatgtcccggccctgtacagcagtgatccagctgcccgggagagggaacgggaagcccgtgaacgagacctccgtgaccgcctcaagcctggctttgaggtgaagcctagtgagctggaacccctacatggggtccctgggccgggcttggatccctttccccgacatgggggcctggctctgcagcctggcccacctggcctgcaccctttcccctttcatccgagcctggggcccctggagcgagaacgtctagcgctggcagctgggccagccctgcggcctgacatgtcctatgctgagcggctggcagctgagaggcagcacgcagaaagggtggcggccctgggcaatgacccactggcccggctgcagatgctcaatgtgactccccatcaccaccagcactcccacatccactcgcacctgcacctgcaccagcaagatgctatccatgcagcctctgcctcggtgcaccctctcattgaccccctggcctcagggtctcaccttacccggatcccctacccagctggaactctccctaaccccctgcttcctcaccctctgcacgagaacgaagttcttcgtcaccagctctttgctgccccttaccgggacctgccggcctccctttctgccccgatgtcagcagctcatcagctgcaggccatgcacgcacagtcagctgagctgcagcgcttggcgctggaacagcagcagtggctgcatgcccatcacccgctgcacagtgtgccgctgcctgcccaggaggactactacagtcacctgaagaaggaaagcgacaagccactgtagaacctgcgatcaagagagcaccatggctcctacattggaccttggagcacccccaccctccccccaccgtgcccttggcctgccacccagagccaagagggtgctgctcagttgcagggcctccgcagctggacagagagtgggggagggagggacagacagaaggccaaggcccgatgtggtgtgcagaggtggggaggtggcgaggatggggacagaaagcgcacagaatcttggaccaggtctctcttccttgtcccccctgcttttctcctcccccatgcccaacccctgtggccgccgcccctcccctgccccgttggtgtgattatttcatctgttagatgtggctgttttgcgtagcatcgtgtgccacccctgcccctccccgatccctgtgtgcgcgccccctctgcaatgtatgccccttgccccttccccacactaataatttatatatataaatatctatatgacgctcttaaaaaaacatcccaaccaaaaccaaccaaacaaaaacatcctcacaactccccaggaa

SEQ ID NO: 472 - DNA, 20 bp, synthetic construct
  misc_feature 1..20: note = Synthetic
  source 1..20: mol_type = other DNA
agagacctggtccaagattc

SEQ ID NO: 473 - DNA, 20 bp, synthetic construct
  source 1..20: mol_type = other DNA
ctcgcgctcgcgctccttct